European Patent Application EP 4 768 507 A1, published July 1, 2026. Title: 双特异性抗体及其应用. Applicant: 合肥天港免疫药物有限公司. Application CN. The sequence listing filed with the application follows.

SEQUENCE LISTING (40 sequences)

SEQ ID NO: 1 - protein, 8 aa, synthetic construct
GFTFNTYA

SEQ ID NO: 2 - protein, 10 aa, synthetic construct
IRSKYNNYAT

SEQ ID NO: 3 - protein, 16 aa, synthetic construct
VRHGNFGNSYVSWFAY

SEQ ID NO: 4 - protein, 9 aa, synthetic construct
TGAVTTSNY

SEQ ID NO: 5 - skipped

SEQ ID NO: 6 - protein, 9 aa, synthetic construct
ALWYSNLWV

SEQ ID NO: 7 - protein, 9 aa, synthetic construct
GFSLTTYGG

SEQ ID NO: 8 - protein, 7 aa, synthetic construct
IWTDGWT

SEQ ID NO: 9 - protein, 13 aa, synthetic construct
ARKGHGYYYAMDY

SEQ ID NO: 10 - protein, 7 aa, synthetic construct
SSVSSSY

SEQ ID NO: 11 - protein, 6 aa, synthetic construct
STSNLI

SEQ ID NO: 12 - protein, 9 aa, synthetic construct
HQYHRSPFT

SEQ ID NO: 13 - protein, 717 aa, synthetic construct
QVQLQESGPGLVKPSETLSLTCTVSGFSLTTYGGHWIRQPPGKGLEWIGMIWTDGWTDYNAAFISRVTISVDTSKNQFSLKLSSVTAADTAVYYCARKGHGYYYAMDYWGQGTLVTVSSASTKGPSVFPLAPSSKSTSGGTAALGCLVKDYFPEPVTVSWNSGALTSGVHTFPAVLQSSGLYSLSSVVTVPSSSLGTQTYICNVNHKPSNTKVDKKVEPKSCDKTHTSPPSPEVQLLESGGGLVQPGGSLKLSCAASGFTFNTYAMNWVRQAPGKGLEWVARIRSKYNNYATYYADSVKDRFTISRDDSKNTAYLQMNNLKTEDTAVYYCVRHGNFGNSYVSWFAYWGQGTLVTVSSGGGGSGGGGSGGGGSELVVTQEPSLTVSPGGTVTLTCRSSTGAVTTSNYANWVQQKPGQAPRGLIGGTNKRAPGTPARFSGSLLGGKAALTLSGVQPEDEAEYYCALWYSNLWVFGGGTKLTVLGGGGSPKSSDKTHTCPPCPAPEAAGGPSVFLFPPKPKDTLMISRTPEVTCVVVDVSHEDPEVKFNWYVDGVEVHNAKTKPREEQYNSTYRVVSVLTVLHQDWLNGKEYKCKVSNKALPAPIEKTISKAKGQPREPQVYTLPPCREEMTKNQVSLWCLVKGFYPSDIAVEWESNGQPENNYKTTPPVLDSDGSFFLYSKLTVDKSRWQQGNVFSCSVMHEALHNHYTQKSLSLSPGK

SEQ ID NO: 14 - protein, 449 aa, synthetic construct
QVQLQESGPGLVKPSETLSLTCTVSGFSLTTYGGHWIRQPPGKGLEWIGMIWTDGWTDYNAAFISRVTISVDTSKNQFSLKLSSVTAADTAVYYCARKGHGYYYAMDYWGQGTLVTVSSASTKGPSVFPLAPSSKSTSGGTAALGCLVKDYFPEPVTVSWNSGALTSGVHTFPAVLQSSGLYSLSSVVTVPSSSLGTQTYICNVNHKPSNTKVDKKVEPKSCDKTHTCPPCPAPEAAGGPSVFLFPPKPKDTLMISRTPEVTCVVVDVSHEDPEVKFNWYVDGVEVHNAKTKPREEQYNSTYRVVSVLTVLHQDWLNGKEYKCKVSNKALPAPIEKTISKAKGQPREPQVCTLPPSREEMTKNQVSLSCAVKGFYPSDIAVEWESNGQPENNYKTTPPVLDSDGSFFLVSKLTVDKSRWQQGNVFSCSVMHEALHNHYTQKSLSLSPGK

SEQ ID NO: 15 - protein, 215 aa, synthetic construct
EIVLTQSPGTLSLSPGERATLSCTASSSVSSSYLHWYQQKPGQAPRLLIYSTSNLISGIPDRFSGSGSGTDFTLTISRLEPEDFAVYYCHQYHRSPFTFGQGTKLEIKRTVAAPSVFIFPPSDEQLKSGTASVVCLLNNFYPREAKVQWKVDNALQSGNSQESVTEQDSKDSTYSLSSTLTLSKADYEKHKVYACEVTHQGLSSPVTKSFNRGEC

SEQ ID NO: 16 - protein, 485 aa, synthetic construct
EVQLLESGGGLVQPGGSLKLSCAASGFTFNTYAMNWVRQAPGKGLEWVARIRSKYNNYATYYADSVKDRFTISRDDSKNTAYLQMNNLKTEDTAVYYCVRHGNFGNSYVSWFAYWGQGTLVTVSSGGGGSGGGGSGGGGSELVVTQEPSLTVSPGGTVTLTCRSSTGAVTTSNYANWVQQKPGQAPRGLIGGTNKRAPGTPARFSGSLLGGKAALTLSGVQPEDEAEYYCALWYSNLWVFGGGTKLTVLGGGGSPKSSDKTHTCPPCPAPEAAGGPSVFLFPPKPKDTLMISRTPEVTCVVVDVSHEDPEVKFNWYVDGVEVHNAKTKPREEQYNSTYRVVSVLTVLHQDWLNGKEYKCKVSNKALPAPIEKTISKAKGQPREPQVYTLPPCREEMTKNQVSLWCLVKGFYPSDIAVEWESNGQPENNYKTTPPVLDSDGSFFLYSKLTVDKSRWQQGNVFSCSVMHEALHNHYTQKSLSLSPGK

SEQ ID NO: 17 - protein, 480 aa, synthetic construct
EVQLVESGGGLVQPGGSLRLSCAASGYSFTGYTMNWVRQAPGKGLEWVALINPYKGVSTYNQKFKDRFTISVDKSKNTAYLQMNSLRAEDTAVYYCARSGYYGDSDWYFDVWGQGTLVTVSSGGGGSGGGGSGGGGSDIQMTQSPSSLSASVGDRVTITCRASQDIRNYLNWYQQKPGKAPKLLIYYTSRLESGVPSRFSGSGSGTDYTLTISSLQPEDFATYYCQQGNTLPWTFGQGTKVEIKGGGGSPKSSDKTHTCPPCPAPEAAGGPSVFLFPPKPKDTLMISRTPEVTCVVVDVSHEDPEVKFNWYVDGVEVHNAKTKPREEQYNSTYRVVSVLTVLHQDWLNGKEYKCKVSNKALPAPIEKTISKAKGQPREPQVYTLPPCREEMTKNQVSLWCLVKGFYPSDIAVEWESNGQPENNYKTTPPVLDSDGSFFLYSKLTVDKSRWQQGNVFSCSVMHEALHNHYTQKSLSLSPGK

SEQ ID NO: 18 - protein, 712 aa, synthetic construct
QVQLQESGPGLVKPSETLSLTCTVSGFSLTTYGGHWIRQPPGKGLEWIGMIWTDGWTDYNAAFISRVTISVDTSKNQFSLKLSSVTAADTAVYYCARKGHGYYYAMDYWGQGTLVTVSSASTKGPSVFPLAPSSKSTSGGTAALGCLVKDYFPEPVTVSWNSGALTSGVHTFPAVLQSSGLYSLSSVVTVPSSSLGTQTYICNVNHKPSNTKVDKKVEPKSCDKTHTSPPSPEVQLVESGGGLVQPGGSLRLSCAASGYSFTGYTMNWVRQAPGKGLEWVALINPYKGVSTYNQKFKDRFTISVDKSKNTAYLQMNSLRAEDTAVYYCARSGYYGDSDWYFDVWGQGTLVTVSSGGGGSGGGGSGGGGSDIQMTQSPSSLSASVGDRVTITCRASQDIRNYLNWYQQKPGKAPKLLIYYTSRLESGVPSRFSGSGSGTDYTLTISSLQPEDFATYYCQQGNTLPWTFGQGTKVEIKGGGGSPKSSDKTHTCPPCPAPEAAGGPSVFLFPPKPKDTLMISRTPEVTCVVVDVSHEDPEVKFNWYVDGVEVHNAKTKPREEQYNSTYRVVSVLTVLHQDWLNGKEYKCKVSNKALPAPIEKTISKAKGQPREPQVYTLPPCREEMTKNQVSLWCLVKGFYPSDIAVEWESNGQPENNYKTTPPVLDSDGSFFLYSKLTVDKSRWQQGNVFSCSVMHEALHNHYTQKSLSLSPGK

SEQ ID NO: 19 - protein, 726 aa, synthetic construct
QVQLQESGPGLVKPSETLSLTCTVSGFSLTTYGGHWIRQPPGKGLEWIGMIWTDGWTDYNAAFISRVTISVDTSKNQFSLKLSSVTAADTAVYYCARKGHGYYYAMDYWGQGTLVTVSSASTKGPSVFPLAPSSKSTSGGTAALGCLVKDYFPEPVTVSWNSGALTSGVHTFPAVLQSSGLYSLSSVVTVPSSSLGTQTYICNVNHKPSNTKVDKKVEPKSCDKTHTSPPSPQAVVTQEPSLTVSPGGTVTLTCRSSTGAVTTSNYANWVQQKPGQAPRGLIGGTNKRAPWTPARFSGSLLGDKAALTITGAQAEDEAEYFCALWYSNLWVFGGGTKLTVLGGSGGSGGSGGSGGSGGSGGSGGSEVQLVESGGGLVQPGGSLKLSCAASGFTFNTYAMNWVRQAPGKGLEWVARIRSKYNNYATYYADSVKDRFTISRDDSKSTLYLQMNSLKTEDTAVYYCVRHGNFGNSYVSWFAYWGQGTLVTVSSGGGGSPKSSDKTHTCPPCPAPEAAGGPSVFLFPPKPKDTLMISRTPEVTCVVVDVSHEDPEVKFNWYVDGVEVHNAKTKPREEQYNSTYRVVSVLTVLHQDWLNGKEYKCKVSNKALPAPIEKTISKAKGQPREPQVYTLPPCREEMTKNQVSLWCLVKGFYPSDIAVEWESNGQPENNYKTTPPVLDSDGSFFLYSKLTVDKSRWQQGNVFSCSVMHEALHNHYTQKSLSLSPGK

SEQ ID NO: 20 - protein, 447 aa, synthetic construct
EIQLVQSGAEVKKPGASVKVSCKASGYAFTSQNIYWVRQAPGQGLEWIGYIEPYNVVPMYNPKFKGRATLTVDKSTSTAYLELSSLRSEDTAVYYCARSGSSNFDYWGQGTLVTVSSASTKGPSVFPLAPSSKSTSGGTAALGCLVKDYFPEPVTVSWNSGALTSGVHTFPAVLQSSGLYSLSSVVTVPSSSLGTQTYICNVNHKPSNTKVDKKVEPKSCDKTHTCPPCPAPEAAGGPSVFLFPPKPKDTLMISRTPEVTCVVVDVSHEDPEVKFNWYVDGVEVHNAKTKPREEQYNSTYRVVSVLTVLHQDWLNGKEYKCKVSNKALPAPIEKTISKAKGQPREPQVCTLPPSREEMTKNQVSLSCAVKGFYPSDIAVEWESNGQPENNYKTTPPVLDSDGSFFLVSKLTVDKSRWQQGNVFSCSVMHEALHNHYTQKSLSLSPGK

SEQ ID NO: 21 - protein, 215 aa, synthetic construct
DIQLTQSPSSLSASVGDRVTITCSASSSISSHYLHWYQQKPGKSPKLLIYRTSNLASGVPSRFSGSGSGTDYTLTISSLQPEDFATYYCQQGSSLPLTFGQGTKVEIKRTVAAPSVFIFPPSDEQLKSGTASVVCLLNNFYPREAKVQWKVDNALQSGNSQESVTEQDSKDSTYSLSSTLTLSKADYEKHKVYACEVTHQGLSSPVTKSFNRGEC

SEQ ID NO: 22 - protein, 715 aa, synthetic construct
EIQLVQSGAEVKKPGASVKVSCKASGYAFTSQNIYWVRQAPGQGLEWIGYIEPYNVVPMYNPKFKGRATLTVDKSTSTAYLELSSLRSEDTAVYYCARSGSSNFDYWGQGTLVTVSSASTKGPSVFPLAPSSKSTSGGTAALGCLVKDYFPEPVTVSWNSGALTSGVHTFPAVLQSSGLYSLSSVVTVPSSSLGTQTYICNVNHKPSNTKVDKKVEPKSCDKTHTSPPSPEVQLLESGGGLVQPGGSLKLSCAASGFTFNTYAMNWVRQAPGKGLEWVARIRSKYNNYATYYADSVKDRFTISRDDSKNTAYLQMNNLKTEDTAVYYCVRHGNFGNSYVSWFAYWGQGTLVTVSSGGGGSGGGGSGGGGSELVVTQEPSLTVSPGGTVTLTCRSSTGAVTTSNYANWVQQKPGQAPRGLIGGTNKRAPGTPARFSGSLLGGKAALTLSGVQPEDEAEYYCALWYSNLWVFGGGTKLTVLGGGGSPKSSDKTHTCPPCPAPEAAGGPSVFLFPPKPKDTLMISRTPEVTCVVVDVSHEDPEVKFNWYVDGVEVHNAKTKPREEQYNSTYRVVSVLTVLHQDWLNGKEYKCKVSNKALPAPIEKTISKAKGQPREPQVYTLPPCREEMTKNQVSLWCLVKGFYPSDIAVEWESNGQPENNYKTTPPVLDSDGSFFLYSKLTVDKSRWQQGNVFSCSVMHEALHNHYTQKSLSLSPGK

SEQ ID NO: 23 - protein, 447 aa, synthetic construct
EVQLVQSGAEVKKPGASVKVSCKASGYAFTNYLIEWVRQAPGQGLEWIGAINPGSGATNYNEKFKDRATLTADKSTNTAYLELSSLRSEDTAVYFCARFLGNYFDNWGQGTLVTVSSASTKGPSVFPLAPSSKSTSGGTAALGCLVKDYFPEPVTVSWNSGALTSGVHTFPAVLQSSGLYSLSSVVTVPSSSLGTQTYICNVNHKPSNTKVDKKVEPKSCDKTHTCPPCPAPEAAGGPSVFLFPPKPKDTLMISRTPEVTCVVVDVSHEDPEVKFNWYVDGVEVHNAKTKPREEQYNSTYRVVSVLTVLHQDWLNGKEYKCKVSNKALPAPIEKTISKAKGQPREPQVCTLPPSREEMTKNQVSLSCAVKGFYPSDIAVEWESNGQPENNYKTTPPVLDSDGSFFLVSKLTVDKSRWQQGNVFSCSVMHEALHNHYTQKSLSLSPGK

SEQ ID NO: 24 - protein, 214 aa, synthetic construct
DIQMTQSPSSLSASVGDRVTITCRASGNIHSYLAWYQQKPGKSPKLLVYYAETLADGVPSRFSGSGSGTDYTLTISSLQPEDFATYFCQQFWTTPYTFGQGTKVEIKRTVAAPSVFIFPPSDEQLKSGTASVVCLLNNFYPREAKVQWKVDNALQSGNSQESVTEQDSKDSTYSLSSTLTLSKADYEKHKVYACEVTHQGLSSPVTKSFNRGEC

SEQ ID NO: 25 - protein, 715 aa, synthetic construct
EVQLVQSGAEVKKPGASVKVSCKASGYAFTNYLIEWVRQAPGQGLEWIGAINPGSGATNYNEKFKDRATLTADKSTNTAYLELSSLRSEDTAVYFCARFLGNYFDNWGQGTLVTVSSASTKGPSVFPLAPSSKSTSGGTAALGCLVKDYFPEPVTVSWNSGALTSGVHTFPAVLQSSGLYSLSSVVTVPSSSLGTQTYICNVNHKPSNTKVDKKVEPKSCDKTHTSPPSPEVQLLESGGGLVQPGGSLKLSCAASGFTFNTYAMNWVRQAPGKGLEWVARIRSKYNNYATYYADSVKDRFTISRDDSKNTAYLQMNNLKTEDTAVYYCVRHGNFGNSYVSWFAYWGQGTLVTVSSGGGGSGGGGSGGGGSELVVTQEPSLTVSPGGTVTLTCRSSTGAVTTSNYANWVQQKPGQAPRGLIGGTNKRAPGTPARFSGSLLGGKAALTLSGVQPEDEAEYYCALWYSNLWVFGGGTKLTVLGGGGSPKSSDKTHTCPPCPAPEAAGGPSVFLFPPKPKDTLMISRTPEVTCVVVDVSHEDPEVKFNWYVDGVEVHNAKTKPREEQYNSTYRVVSVLTVLHQDWLNGKEYKCKVSNKALPAPIEKTISKAKGQPREPQVYTLPPCREEMTKNQVSLWCLVKGFYPSDIAVEWESNGQPENNYKTTPPVLDSDGSFFLYSKLTVDKSRWQQGNVFSCSVMHEALHNHYTQKSLSLSPGK

SEQ ID NO: 26 - protein, 451 aa, synthetic construct
QVQLVESGGGLVKPGGSLRLSCAASGFTFSNYAMSWIRQAPGKGLEWVSYISPGGDYIYYADSVKGRFTISRDNAKNSLYLQMNSLRAEDTAVYYCTTDRRHYGSYAMDYWGQGTLVTVSSASTKGPSVFPLAPSSKSTSGGTAALGCLVKDYFPEPVTVSWNSGALTSGVHTFPAVLQSSGLYSLSSVVTVPSSSLGTQTYICNVNHKPSNTKVDKKVEPKSCDKTHTCPPCPAPEAAGGPSVFLFPPKPKDTLMISRTPEVTCVVVDVSHEDPEVKFNWYVDGVEVHNAKTKPREEQYNSTYRVVSVLTVLHQDWLNGKEYKCKVSNKALPAPIEKTISKAKGQPREPQVCTLPPSREEMTKNQVSLSCAVKGFYPSDIAVEWESNGQPENNYKTTPPVLDSDGSFFLVSKLTVDKSRWQQGNVFSCSVMHEALHNHYTQKSLSLSPGK

SEQ ID NO: 27 - protein, 219 aa, synthetic construct
DIVMTQSPLSLPVTPGEPASISCRSSKSLLHSNLNTYLYWFLQKPGQSPQILIYRMSNLASGVPDRFSGSGSGTAFTLKISRVEAEDVGVYYCMQHLEYPFTFGPGTKLEIKRTVAAPSVFIFPPSDEQLKSGTASVVCLLNNFYPREAKVQWKVDNALQSGNSQESVTEQDSKDSTYSLSSTLTLSKADYEKHKVYACEVTHQGLSSPVTKSFNRGEC

SEQ ID NO: 28 - protein, 719 aa, synthetic construct
QVQLVESGGGLVKPGGSLRLSCAASGFTFSNYAMSWIRQAPGKGLEWVSYISPGGDYIYYADSVKGRFTISRDNAKNSLYLQMNSLRAEDTAVYYCTTDRRHYGSYAMDYWGQGTLVTVSSASTKGPSVFPLAPSSKSTSGGTAALGCLVKDYFPEPVTVSWNSGALTSGVHTFPAVLQSSGLYSLSSVVTVPSSSLGTQTYICNVNHKPSNTKVDKKVEPKSCDKTHTSPPSPEVQLLESGGGLVQPGGSLKLSCAASGFTFNTYAMNWVRQAPGKGLEWVARIRSKYNNYATYYADSVKDRFTISRDDSKNTAYLQMNNLKTEDTAVYYCVRHGNFGNSYVSWFAYWGQGTLVTVSSGGGGSGGGGSGGGGSELVVTQEPSLTVSPGGTVTLTCRSSTGAVTTSNYANWVQQKPGQAPRGLIGGTNKRAPGTPARFSGSLLGGKAALTLSGVQPEDEAEYYCALWYSNLWVFGGGTKLTVLGGGGSPKSSDKTHTCPPCPAPEAAGGPSVFLFPPKPKDTLMISRTPEVTCVVVDVSHEDPEVKFNWYVDGVEVHNAKTKPREEQYNSTYRVVSVLTVLHQDWLNGKEYKCKVSNKALPAPIEKTISKAKGQPREPQVYTLPPCREEMTKNQVSLWCLVKGFYPSDIAVEWESNGQPENNYKTTPPVLDSDGSFFLYSKLTVDKSRWQQGNVFSCSVMHEALHNHYTQKSLSLSPGK

SEQ ID NO: 29 - protein, 119 aa, synthetic construct
QVQLQESGPGLVKPSETLSLTCTVSGFSLTTYGGHWIRQPPGKGLEWIGMIWTDGWTDYNAAFISRVTISVDTSKNQFSLKLSSVTAADTAVYYCARKGHGYYYAMDYWGQGTLVTVSS

SEQ ID NO: 30 - protein, 108 aa, synthetic construct
EIVLTQSPGTLSLSPGERATLSCTASSSVSSSYLHWYQQKPGQAPRLLIYSTSNLISGIPDRFSGSGSGTDFTLTISRLEPEDFAVYYCHQYHRSPFTFGQGTKLEIK

SEQ ID NO: 31 - protein, 218 aa, synthetic construct
QVQLQESGPGLVKPSETLSLTCTVSGFSLTTYGGHWIRQPPGKGLEWIGMIWTDGWTDYNAAFISRVTISVDTSKNQFSLKLSSVTAADTAVYYCARKGHGYYYAMDYWGQGTLVTVSSASTKGPSVFPLAPSSKSTSGGTAALGCLVKDYFPEPVTVSWNSGALTSGVHTFPAVLQSSGLYSLSSVVTVPSSSLGTQTYICNVNHKPSNTKVDKKVE

SEQ ID NO: 32 - protein, 215 aa, synthetic construct; identical to SEQ ID NO: 15

SEQ ID NO: 33 - protein, 125 aa, synthetic construct
EVQLLESGGGLVQPGGSLKLSCAASGFTFNTYAMNWVRQAPGKGLEWVARIRSKYNNYATYYADSVKDRFTISRDDSKNTAYLQMNNLKTEDTAVYYCVRHGNFGNSYVSWFAYWGQGTLVTVSS

SEQ ID NO: 34 - protein, 109 aa, synthetic construct
ELVVTQEPSLTVSPGGTVTLTCRSSTGAVTTSNYANWVQQKPGQAPRGLIGGTNKRAPGTPARFSGSLLGGKAALTLSGVQPEDEAEYYCALWYSNLWVFGGGTKLTVL

SEQ ID NO: 35 - protein, 249 aa, synthetic construct
EVQLLESGGGLVQPGGSLKLSCAASGFTFNTYAMNWVRQAPGKGLEWVARIRSKYNNYATYYADSVKDRFTISRDDSKNTAYLQMNNLKTEDTAVYYCVRHGNFGNSYVSWFAYWGQGTLVTVSSGGGGSGGGGSGGGGSELVVTQEPSLTVSPGGTVTLTCRSSTGAVTTSNYANWVQQKPGQAPRGLIGGTNKRAPGTPARFSGSLLGGKAALTLSGVQPEDEAEYYCALWYSNLWVFGGGTKLTVL

SEQ ID NO: 36 - protein, 5 aa, synthetic construct
GGGGS

SEQ ID NO: 37 - protein, 15 aa, synthetic construct
GGGGSGGGGSGGGGS

SEQ ID NO: 38 - protein, 231 aa, synthetic construct
PKSSDKTHTCPPCPAPEAAGGPSVFLFPPKPKDTLMISRTPEVTCVVVDVSHEDPEVKFNWYVDGVEVHNAKTKPREEQYNSTYRVVSVLTVLHQDWLNGKEYKCKVSNKALPAPIEKTISKAKGQPREPQVYTLPPCREEMTKNQVSLWCLVKGFYPSDIAVEWESNGQPENNYKTTPPVLDSDGSFFLYSKLTVDKSRWQQGNVFSCSVMHEALHNHYTQKSLSLSPGK

SEQ ID NO: 39 - protein, 231 aa, synthetic construct
PKSCDKTHTCPPCPAPEAAGGPSVFLFPPKPKDTLMISRTPEVTCVVVDVSHEDPEVKFNWYVDGVEVHNAKTKPREEQYNSTYRVVSVLTVLHQDWLNGKEYKCKVSNKALPAPIEKTISKAKGQPREPQVCTLPPSREEMTKNQVSLSCAVKGFYPSDIAVEWESNGQPENNYKTTPPVLDSDGSFFLVSKLTVDKSRWQQGNVFSCSVMHEALHNHYTQKSLSLSPGK

SEQ ID NO: 40 - protein, 231 aa, synthetic construct
PKSSDKTHTCPPCPAPEAAGGPSVFLFPPKPKDTLMISRTPEVTCVVVDVSHEDPEVKFNWYVDGVEVHNAKTKPREEQYNSTYRVVSVLTVLHQDWLNGKEYKCKVSNKALPAPIEKTISKAKGQPREPQVCTLPPSREEMTKNQVSLSCAVKGFYPSDIAVEWESNGQPENNYKTTPPVLDSDGSFFLVSKLTVDKSRWQQGNVFSCSVMHEALHNHYTQKSLSLSPGK